European Patent Specification EP 4 026 543 B1, published August 7, 2024. Title: Polymer Protein Microparticles. Applicant: Regeneron Pharmaceuticals, Inc. Application EP19180351.9. The sequence listing filed with the application follows.

SEQUENCE LISTING (1 sequence)

SEQ ID NO: 1 - protein, 415 aa, Artificial Sequence
  synthetic
IIHMTEGRELVIPCRVTSPNITVTLKKFPLDTLIPDGKRIIWDSRKGFIISNATYKEIGLLTCEATVNGHLYKTNYLTHRQTNTIIDVVLSPSHGIELSVGEKLVLNCTARTELNVGIDFNWEYPSSKHQHKKLVNRDLKTQSGSEMKKFLSTLTIDGVTRSDQGLYTCAASSGLMTKKNSTFVRVHEKDKTHTCPPCPAPELLGGPSVFLFPPKPKDTLMISRTPEVTCVVVDVSHEDPEVKFNWYVDGVEVHNAKTKPREEQYNSTYRVVSVLTVLHQDWLNGKEYKCKVSNKALPAPIEKTISKAKGQPREPQVYTLPPSRDELTKNQVSLTCLVKGFYPSDIAVEWESNGQPENNYKTTPPVLDSDGSFFLYSKLTVDKSRWQQGNVFSCSVMHEALHNHYTQKSLSLSPG